European Patent Application EP 4 446 404 A1, published October 16, 2024. Title: COMPOSITION FOR PREVENTING OR TREATING COGNITIVE DISORDER AND INTESTINAL DISORDER COMPRISING LACTOBACILLUS PARACASEI NK112, CUSCUTA CHINENSIS LAM EXTRACT AND CUSCUTA JAPONICA CHOISY EXTRACT. Applicant: MThera Pharma Co., Ltd. University-Industry Cooperation Group of Kyung Hee University Gachon University of Industry-Academic cooperation Foundation Konkuk University Industrial Cooperation Corp. The sequence listing filed with the application follows.

SEQUENCE LISTING (1 sequence)

SEQ ID NO: 1 - DNA, 1380 bp, Artificial Sequence
  NK112
acctgcccttaagtgggggataacatttggaaacagatgctaataccgcatagatccaagaaccgcatggttcttggctgaaagatggcgtaagctatcgcttttggatggacccgcggcgtattagctagttggtgaggtaatggctcaccaaggcgatgatacgtagccgaactgagaggttgatcggccacattgggactgagacacggcccaaactcctacgggaggcagcagtagggaatcttccacaatggacgcaagtctgatggagcaacgccgcgtgagtgaagaaggctttcgggtcgtaaaactctgttgttggagaagaatggtcggcagagtaactgttgtcggcgtgacggtatccaaccagaaagccacggctaactacgtgccagcagccgcggtaatacgtaggtggcaagcgttatccggatttattgggcgtaaagcgagcgcaggcggttttttaagtctgatgtgaaagccctcggcttaaccgaggaagcgcatcggaaactgggaaacttgagtgcagaagaggacagtggaactccatgtgtagcggtgaaatgcgtagatatatggaagaacaccagtggcgaaggcggctgtctggtctgtaactgacgctgaggctcgaaagcatgggtagcgaacaggattagataccctggtagtccatgccgtaaacgatgaatgctaggtgttggagggtttccgcccttcagtgccgcagctaacgcattaagcattccgcctggggagtacgaccgcaaggttgaaactcaaaggaattgacgggggcccgcacaagcggtggagcatgtggtttaattcgaagcaacgcgaagaaccttaccaggtcttgacatcttttgatcacctgagagatcaggtttccccttcgggggcaaaatgacaggtggtgcatggttgtcgtcagctcgtgtcgtgagatgttgggttaagtcccgcaacgagcgcaacccttatgactagttgccagcatttagttgggcactctagtaagactgccggtgacaaaccggaggaaggtggggatgacgtcaaatcatcatgccccttatgacctgggctacacacgtgctacaatggatggtacaacgagttgcgagaccgcgaggtcaagctaatctcttaaagccattctcagttcggactgtaggctgcaactcgcctacacgaagtcggaatcgctagtaatcgcggatcagcacgccgcggtgaatacgttcccgggccttgtacacaccgcccgtcacaccatgagagtttgtaacacccgaagccggtggcgtaacccttttagggagcgagccgtctaaggtgggacaatgattagggtgaagtcta